European Patent Application EP 4 282 969 A2, published November 29, 2023. Title: COMPOSITIONS AND METHODS FOR TREATING CANCER WITH DUOCARS. Applicant: Lentigen Technology, Inc. Application EP 23184693.2, filed September 1, 2017. The sequence listing filed with the application follows.

SEQUENCE LISTING (55 sequences)

SEQ ID NO: 1 - DNA, 729 bp, synthetic construct
  misc_feature 1..729: note = CD20-reactive scFv binding domain
  source 1..729: mol_type = other DNA
gaggtgcagttgcaacagtcaggagctgaactggtcaagccaggagccagcgtgaagatgagctgcaaggcctccggttacaccttcacctcctacaacatgcactgggtgaaacagaccccgggacaagggctcgaatggattggcgccatctaccccgggaatggcgatacttcgtacaaccagaagttcaagggaaaggccaccctgaccgccgacaagagctcctccaccgcgtatatgcagttgagctccctgacctccgaggactccgccgactactactgcgcacggtccaactactatggaagctcgtactggttcttcgatgtctggggggccggcaccactgtgaccgtcagctccgggggcggaggatccggtggaggcggaagcgggggtggaggatccgacattgtgctgactcagtccccggcaatcctgtcggcctcaccgggcgaaaaggtcacgatgacttgtagagcgtcgtccagcgtgaactacatggattggtaccaaaagaagcctggatcgtcacccaagccttggatctacgctacatctaacctggcctccggcgtgccagcgcggttcagcgggtccggctcgggcacctcatactcgctgaccatctcccgcgtggaggctgaggacgccgcgacctactactgccagcagtggtccttcaacccgccgacttttggaggcggtactaagctggagatcaaa

SEQ ID NO: 2 - protein, 243 aa, synthetic construct
  REGION 1..243: note = CD20-reactive scFv binding domain
EVQLQQSGAELVKPGASVKMSCKASGYTFTSYNMHWVKQTPGQGLEWIGAIYPGNGDTSYNQKFKGKATLTADKSSSTAYMQLSSLTSEDSADYYCARSNYYGSSYWFFDVWGAGTTVTVSSGGGGSGGGGSGGGGSDIVLTQSPAILSASPGEKVTMTCRASSSVNYMDWYQKKPGSSPKPWIYATSNLASGVPARFSGSGSGTSYSLTISRVEAEDAATYYCQQWSFNPPTFGGGTKLEIK

SEQ ID NO: 3 - DNA, 1473 bp, synthetic construct
  misc_feature 1..1473: note = LP-1495-CD8 TM-41BB-CD3zeta
  source 1..1473: mol_type = other DNA
atgctccttctcgtgacctccctgcttctctgcgaactgccccatcctgccttcctgctgattcccgaggtgcagttgcaacagtcaggagctgaactggtcaagccaggagccagcgtgaagatgagctgcaaggcctccggttacaccttcacctcctacaacatgcactgggtgaaacagaccccgggacaagggctcgaatggattggcgccatctaccccgggaatggcgatacttcgtacaaccagaagttcaagggaaaggccaccctgaccgccgacaagagctcctccaccgcgtatatgcagttgagctccctgacctccgaggactccgccgactactactgcgcacggtccaactactatggaagctcgtactggttcttcgatgtctggggggccggcaccactgtgaccgtcagctccgggggcggaggatccggtggaggcggaagcgggggtggaggatccgacattgtgctgactcagtccccggcaatcctgtcggcctcaccgggcgaaaaggtcacgatgacttgtagagcgtcgtccagcgtgaactacatggattggtaccaaaagaagcctggatcgtcacccaagccttggatctacgctacatctaacctggcctccggcgtgccagcgcggttcagcgggtccggctcgggcacctcatactcgctgaccatctcccgcgtggaggctgaggacgccgcgacctactactgccagcagtggtccttcaacccgccgacttttggaggcggtactaagctggagatcaaagcggccgcaactaccacccctgcccctcggccgccgactccggccccaaccatcgcaagccaacccctctccttgcgccccgaagcttgccgcccggccgcgggtggagccgtgcatacccgggggctggactttgcctgcgatatctacatttgggccccgctggccggcacttgcggcgtgctcctgctgtcgctggtcatcaccctttactgcaagaggggccggaagaagctgctttacatcttcaagcagccgttcatgcggcccgtgcagacgactcaggaagaggacggatgctcgtgcagattccctgaggaggaagaggggggatgcgaactgcgcgtcaagttctcacggtccgccgacgcccccgcatatcaacagggccagaatcagctctacaacgagctgaacctgggaaggagagaggagtacgacgtgctggacaagcgacgcggacgcgacccggagatgggggggaaaccacggcggaaaaaccctcaggaaggactgtacaacgaactccagaaagacaagatggcggaagcctactcagaaatcgggatgaagggagagcggaggaggggaaagggtcacgacgggctgtaccagggactgagcaccgccactaaggatacctacgatgccttgcatatgcaagcactcccaccccgg

SEQ ID NO: 4 - protein, 491 aa, synthetic construct
  REGION 1..491: note = LP-1495-CD8 TM-41BB-CD3zeta
MLLLVTSLLLCELPHPAFLLIPEVQLQQSGAELVKPGASVKMSCKASGYTFTSYNMHWVKQTPGQGLEWIGAIYPGNGDTSYNQKFKGKATLTADKSSSTAYMQLSSLTSEDSADYYCARSNYYGSSYWFFDVWGAGTTVTVSSGGGGSGGGGSGGGGSDIVLTQSPAILSASPGEKVTMTCRASSSVNYMDWYQKKPGSSPKPWIYATSNLASGVPARFSGSGSGTSYSLTISRVEAEDAATYYCQQWSFNPPTFGGGTKLEIKAAATTTPAPRPPTPAPTIASQPLSLRPEACRPAAGGAVHTRGLDFACDIYIWAPLAGTCGVLLLSLVITLYCKRGRKKLLYIFKQPFMRPVQTTQEEDGCSCRFPEEEEGGCELRVKFSRSADAPAYQQGQNQLYNELNLGRREEYDVLDKRRGRDPEMGGKPRRKNPQEGLYNELQKDKMAEAYSEIGMKGERRRGKGHDGLYQGLSTATKDTYDALHMQALPPR

SEQ ID NO: 5 - DNA, 66 bp, synthetic construct
  misc_feature 1..66: note = leader/signal peptide sequence
  source 1..66: mol_type = other DNA
atgctgctgctggtgaccagcctgctgctgtgcgaactgccgcatccggcgtttctgctgattccg

SEQ ID NO: 6 - protein, 22 aa, synthetic construct
  REGION 1..22: note = leader/signal peptide sequence
MLLLVTSLLLCELPHPAFLLIP

SEQ ID NO: 7 - DNA, 747 bp, synthetic construct
  misc_feature 1..747: note = CD22-reactive scFv binding domain
  source 1..747: mol_type = other DNA
caggtacagctccagcagagtggcccagggctcgtgaagccaagccagacgctgtccctgacttgtgcaatttcaggggattcagtttcatcaaatagcgcggcgtggaattggattcgacaatctccttcccgagggttggaatggcttggacgaacatattacagatccaaatggtataacgactatgcggtatcagtaaagtcaagaataaccattaaccccgacacaagcaagaaccaattctctttgcagcttaactctgtcacgccagaagacacggcagtctattattgcgctcgcgaggtaacgggtgacctggaagacgcttttgacatttgggggcagggtacgatggtgacagtcagttcagggggcggtgggagtgggggagggggtagcggggggggagggtcagacattcagatgacccagtccccttcatccttgtctgcctccgtcggtgacagggtgacaataacatgcagagcaagccaaacaatctggagctatctcaactggtaccagcagcgaccaggaaaagcgccaaacctgctgatttacgctgcttcctccctccaatcaggcgtgcctagtagatttagcggtaggggctccggcaccgattttacgctcactataagctctcttcaagcagaagattttgcgacttattactgccagcagtcctatagtatacctcagactttcggacagggtaccaagttggagattaaggcggccgca

SEQ ID NO: 8 - protein, 249 aa, synthetic construct
  REGION 1..249: note = CD22-reactive scFv binding domain
QVQLQQSGPGLVKPSQTLSLTCAISGDSVSSNSAAWNWIRQSPSRGLEWLGRTYYRSKWYNDYAVSVKSRITINPDTSKNQFSLQLNSVTPEDTAVYYCAREVTGDLEDAFDIWGQGTMVTVSSGGGGSGGGGSGGGGSDIQMTQSPSSLSASVGDRVTITCRASQTIWSYLNWYQQRPGKAPNLLIYAASSLQSGVPSRFSGRGSGTDFTLTISSLQAEDFATYYCQQSYSIPQTFGQGTKLEIKAAA

SEQ ID NO: 9 - DNA, 1482 bp, synthetic construct
  misc_feature 1..1482: note = LP-2200-CD8 TM-41BB-CD3zeta
  source 1..1482: mol_type = other DNA
atgcttcttttggtgacttcccttttgctgtgcgagttgccacaccccgccttcctgcttattccccaggtacagctccagcagagtggcccagggctcgtgaagccaagccagacgctgtccctgacttgtgcaatttcaggggattcagtttcatcaaatagcgcggcgtggaattggattcgacaatctccttcccgagggttggaatggcttggacgaacatattacagatccaaatggtataacgactatgcggtatcagtaaagtcaagaataaccattaaccccgacacaagcaagaaccaattctctttgcagcttaactctgtcacgccagaagacacggcagtctattattgcgctcgcgaggtaacgggtgacctggaagacgcttttgacatttgggggcagggtacgatggtgacagtcagttcagggggcggtgggagtgggggagggggtagcggggggggagggtcagacattcagatgacccagtccccttcatccttgtctgcctccgtcggtgacagggtgacaataacatgcagagcaagccaaacaatctggagctatctcaactggtaccagcagcgaccaggaaaagcgccaaacctgctgatttacgctgcttcctccctccaatcaggcgtgcctagtagatttagcggtaggggctccggcaccgattttacgctcactataagctctcttcaagcagaagattttgcgacttattactgccagcagtcctatagtatacctcagactttcggacagggtaccaagttggagattaaggcggccgcaactaccacccctgcccctcggccgccgactccggccccaaccatcgcaagccaacccctctccttgcgccccgaagcttgccgcccggccgcgggtggagccgtgcatacccgggggctggactttgcctgcgatatctacatttgggccccgctggccggcacttgcggcgtgctcctgctgtcgctggtcatcaccctttactgcaagaggggccggaagaagctgctttacatcttcaagcagccgttcatgcggcccgtgcagacgactcaggaagaggacggatgctcgtgcagattccctgaggaggaagaggggggatgcgaactgcgcgtcaagttctcacggtccgccgacgcccccgcatatcaacagggccagaatcagctctacaacgagctgaacctgggaaggagagaggagtacgacgtgctggacaagcgacgcggacgcgacccggagatgggggggaaaccacggcggaaaaaccctcaggaaggactgtacaacgaactccagaaagacaagatggcggaagcctactcagaaatcgggatgaagggagagcggaggaggggaaagggtcacgacgggctgtaccagggactgagcaccgccactaaggatacctacgatgccttgcatatgcaagcactcccaccccgg

SEQ ID NO: 10 - protein, 494 aa, synthetic construct
  REGION 1..494: note = LP-2200-CD8 TM-41BB-CD3zeta
MLLLVTSLLLCELPHPAFLLIPQVQLQQSGPGLVKPSQTLSLTCAISGDSVSSNSAAWNWIRQSPSRGLEWLGRTYYRSKWYNDYAVSVKSRITINPDTSKNQFSLQLNSVTPEDTAVYYCAREVTGDLEDAFDIWGQGTMVTVSSGGGGSGGGGSGGGGSDIQMTQSPSSLSASVGDRVTITCRASQTIWSYLNWYQQRPGKAPNLLIYAASSLQSGVPSRFSGRGSGTDFTLTISSLQAEDFATYYCQQSYSIPQTFGQGTKLEIKAAATTTPAPRPPTPAPTIASQPLSLRPEACRPAAGGAVHTRGLDFACDIYIWAPLAGTCGVLLLSLVITLYCKRGRKKLLYIFKQPFMRPVQTTQEEDGCSCRFPEEEEGGCELRVKFSRSADAPAYQQGQNQLYNELNLGRREEYDVLDKRRGRDPEMGGKPRRKNPQEGLYNELQKDKMAEAYSEIGMKGERRRGKGHDGLYQGLSTATKDTYDALHMQALPPR

SEQ ID NO: 11 - DNA, 72 bp, Homo sapiens
  source 1..72: mol_type = other DNA
atctacatctgggcgcccttggccgggacttgtggggtccttctcctgtcactggttatcaccctttactgc

SEQ ID NO: 12 - protein, 22 aa, Homo sapiens
IWAPLAGTCGVLLLSLVITLYC

SEQ ID NO: 13 - DNA, 141 bp, Homo sapiens
  source 1..141: mol_type = other DNA
accacgacgccagcgccgcgaccaccaacaccggcgcccaccatcgcgtcgcagcccctgtccctgcgcccagaggcgtgccggccagcggcggggggcgcagtgcacacgagggggctggactttgcctgcgatatctac

SEQ ID NO: 14 - protein, 47 aa, Homo sapiens
TTTPAPRPPTPAPTIASQPLSLRPEACRPAAGGAVHTRGLDFACDIY

SEQ ID NO: 15 - protein, 69 aa, Homo sapiens
TTTPAPRPPTPAPTIASQPLSLRPEACRPAAGGAVHTRGLDFACDIYIWAPLAGTCGVLLLSLVITLYC

SEQ ID NO: 16 - protein, 106 aa, Homo sapiens
GQPKAAPSVTLFPPSSEELQANKATLVCLISDFYPGAVTVAWKADSSPVKAGVETTTPSKQSNNKYAASSYLSLTPEQWKSHRSYSCQVTHEGSTVEKTVAPTECS

SEQ ID NO: 17 - DNA, 126 bp, Homo sapiens
  source 1..126: mol_type = other DNA
aaacggggcagaaagaaactcctgtatatattcaaacaaccatttatgagaccagtacaaactactcaagaggaagatggctgtagctgccgatttccagaagaagaagaaggaggatgtgaactg

SEQ ID NO: 18 - protein, 42 aa, Homo sapiens
KRGRKKLLYIFKQPFMRPVQTTQEEDGCSCRFPEEEEGGCEL

SEQ ID NO: 19 - DNA, 336 bp, synthetic construct
  misc_feature 1..336: note = signaling domain of CD3-zeta
  source 1..336: mol_type = other DNA
agagtgaagttcagcaggagcgcagacgcccccgcgtacaagcagggccagaaccagctctataacgagctcaatctaggacgaagagaggagtacgatgttttggacaagagacgtggccgggaccctgagatggggggaaagccgagaaggaagaaccctcaggaaggcctgtacaatgaactgcagaaagataagatggcggaggcctacagtgagattgggatgaaaggcgagcgccggaggggcaaggggcacgatggcctttaccagggtctcagtacagccaccaaggacacctacgacgcccttcacatgcaggccctgccccctcgc

SEQ ID NO: 20 - protein, 112 aa, Homo sapiens
RVKFSRSADAPAYKQGQNQLYNELNLGRREEYDVLDKRRGRDPEMGGKPRRKNPQEGLYNELQKDKMAEAYSEIGMKGERRRGKGHDGLYQGLSTATKDTYDALHMQALPPR

SEQ ID NO: 21 - DNA, 1467 bp, synthetic construct
  misc_feature 1..1467: note = LP-CD19binder-CD8linker-CD4tm-4-1BB-CD3-zeta
  source 1..1467: mol_type = other DNA
atgctgctgctggtgaccagcctgctgctgtgcgaactgccgcatccggcgtttctgctgattccggatattcagatgacccagaccaccagcagcctgagcgcgagcctgggcgatcgcgtgaccattagctgccgcgcgagccaggatattagcaaatatctgaactggtatcagcagaaaccggatggcaccgtgaaactgctgatttatcataccagccgcctgcatagcggcgtgccgagccgctttagcggcagcggcagcggcaccgattatagcctgaccattagcaacctggaacaggaagatattgcgacctatttttgccagcagggcaacaccctgccgtatacctttggcggcggcaccaaactggaaattaccggcggcggcggcagcggcggcggcggcagcggcggcggcggcagcgaagtgaaactgcaggaaagcggcccgggcctggtggcgccgagccagagcctgagcgtgacctgcaccgtgagcggcgtgagcctgccggattatggcgtgagctggattcgccagccgccgcgcaaaggcctggaatggctgggcgtgatttggggcagcgaaaccacctattataacagcgcgctgaaaagccgcctgaccattattaaagataacagcaaaagccaggtgtttctgaaaatgaacagcctgcagaccgatgataccgcgatttattattgcgcgaaacattattattatggcggcagctatgcgatggattattggggccagggcaccagcgtgaccgtgagcagcgcggcggcgccggcgccgcgcccgccgaccccggcgccgaccattgcgagccagccgctgagcctgcgcccggaagcgtgccgcccggcggcgggcggcgcggtgcatacccgcggcctggattttgtgcagccgatggcgctgattgtgctgggcggcgtggcgggcctgctgctgtttattggcctgggcatttttttttgcgtgcgctgccgcccgcgccgcaaaaaactgctgtatatttttaaacagccgtttatgcgcccggtgcagaccacccaggaagaagatggctgcagctgccgctttccggaagaagaagaaggcggctgcgaactgcgcgtgaaatttagccgcagcgcggatgcgccggcgtatcagcagggccagaaccagctgtataacgaactgaacctgggccgccgcgaagaatatgatgtgctggataaacgccgcggccgcgatccggaaatgggcggcaaaccgcgccgcaaaaacccgcaggaaggcctgtataacgaactgcagaaagataaaatggcggaagcgtatagcgaaattggcatgaaaggcgaacgccgccgcggcaaaggccatgatggcctgtatcagggcctgagcaccgcgaccaaagatacctatgatgcgctgcatatgcaggcgctgccgccgcgc

SEQ ID NO: 22 - protein, 489 aa, synthetic construct
  REGION 1..489: note = LP-CD19binder-CD8linker-CD4tm-4-1BB-CD3-zeta
MLLLVTSLLLCELPHPAFLLIPDIQMTQTTSSLSASLGDRVTISCRASQDISKYLNWYQQKPDGTVKLLIYHTSRLHSGVPSRFSGSGSGTDYSLTISNLEQEDIATYFCQQGNTLPYTFGGGTKLEITGGGGSGGGGSGGGGSEVKLQESGPGLVAPSQSLSVTCTVSGVSLPDYGVSWIRQPPRKGLEWLGVIWGSETTYYNSALKSRLTIIKDNSKSQVFLKMNSLQTDDTAIYYCAKHYYYGGSYAMDYWGQGTSVTVSSAAAPAPRPPTPAPTIASQPLSLRPEACRPAAGGAVHTRGLDFVQPMALIVLGGVAGLLLFIGLGIFFCVRCRPRRKKLLYIFKQPFMRPVQTTQEEDGCSCRFPEEEEGGCELRVKFSRSADAPAYQQGQNQLYNELNLGRREEYDVLDKRRGRDPEMGGKPRRKNPQEGLYNELQKDKMAEAYSEIGMKGERRRGKGHDGLYQGLSTATKDTYDALHMQALPPR

SEQ ID NO: 23 - DNA, 1548 bp, synthetic construct
  misc_feature 1..1548: note = CD20_19-reactive scFv binding domain
  source 1..1548: mol_type = other DNA
gaggtgcagttgcaacagtcaggagctgaactggtcaagccaggagccagcgtgaagatgagctgcaaggcctccggttacaccttcacctcctacaacatgcactgggtgaaacagaccccgggacaagggctcgaatggattggcgccatctaccccgggaatggcgatacttcgtacaaccagaagttcaagggaaaggccaccctgaccgccgacaagagctcctccaccgcgtatatgcagttgagctccctgacctccgaggactccgccgactactactgcgcacggtccaactactatggaagctcgtactggttcttcgatgtctggggggccggcaccactgtgaccgtcagctccgggggcggaggatccggtggaggcggaagcgggggtggaggatccgacattgtgctgactcagtccccggcaatcctgtcggcctcaccgggcgaaaaggtcacgatgacttgtagagcgtcgtccagcgtgaactacatggattggtaccaaaagaagcctggatcgtcacccaagccttggatctacgctacatctaacctggcctccggcgtgccagcgcggttcagcgggtccggctcgggcacctcatactcgctgaccatctcccgcgtggaggctgaggacgccgcgacctactactgccagcagtggtccttcaacccgccgacttttggaggcggtactaagctggagatcaaaggaggcggcggcagcggcgggggagggtccggagggggtggttctggtggaggaggatcgggaggcggtggcagcgacattcagatgactcagaccacctcctccctgtccgcctccctgggcgaccgcgtgaccatctcatgccgcgccagccaggacatctcgaagtacctcaactggtaccagcagaagcccgacggaaccgtgaagctcctgatctaccacacctcccggctgcacagcggagtgccgtctagattctcgggttcggggtcgggaactgactactcccttactatttccaacctggagcaggaggatattgccacctacttctgccaacaaggaaacaccctgccgtacacttttggcgggggaaccaagctggaaatcactggcagcacatccggttccgggaagcccggctccggagagggcagcaccaagggggaagtcaagctgcaggaatcaggacctggcctggtggccccgagccagtcactgtccgtgacttgtactgtgtccggagtgtcgctcccggattacggagtgtcctggatcaggcagccacctcggaaaggattggaatggctcggagtcatctggggttccgaaaccacctattacaactcggcactgaaatccaggctcaccattatcaaggataactccaagtcacaagtgttcctgaagatgaatagcctgcagactgacgacacggcgatctactattgcgccaagcactactactacggcggatcctacgctatggactactggggccaggggaccagcgtgaccgtgtcatccgcggccgca

SEQ ID NO: 24 - protein, 516 aa, synthetic construct
  REGION 1..516: note = CD20_19-reactive scFv binding domain
EVQLQQSGAELVKPGASVKMSCKASGYTFTSYNMHWVKQTPGQGLEWIGAIYPGNGDTSYNQKFKGKATLTADKSSSTAYMQLSSLTSEDSADYYCARSNYYGSSYWFFDVWGAGTTVTVSSGGGGSGGGGSGGGGSDIVLTQSPAILSASPGEKVTMTCRASSSVNYMDWYQKKPGSSPKPWIYATSNLASGVPARFSGSGSGTSYSLTISRVEAEDAATYYCQQWSFNPPTFGGGTKLEIKGGGGSGGGGSGGGGSGGGGSGGGGSDIQMTQTTSSLSASLGDRVTISCRASQDISKYLNWYQQKPDGTVKLLIYHTSRLHSGVPSRFSGSGSGTDYSLTISNLEQEDIATYFCQQGNTLPYTFGGGTKLEITGSTSGSGKPGSGEGSTKGEVKLQESGPGLVAPSQSLSVTCTVSGVSLPDYGVSWIRQPPRKGLEWLGVIWGSETTYYNSALKSRLTIIKDNSKSQVFLKMNSLQTDDTAIYYCAKHYYYGGSYAMDYWGQGTSVTVSSAAA

SEQ ID NO: 25 - DNA, 2283 bp, synthetic construct
  misc_feature 1..2283: note = LP-CD20 VH-(GGGGS)3-CD20 VL-(GGGGS)5-CD19VL-Whitlow linker-CD19 VH-CD8 hinge+TM-41BB-CD3zeta
  source 1..2283: mol_type = other DNA
atgctccttctcgtgacctccctgcttctctgcgaactgccccatcctgccttcctgctgattcccgaggtgcagttgcaacagtcaggagctgaactggtcaagccaggagccagcgtgaagatgagctgcaaggcctccggttacaccttcacctcctacaacatgcactgggtgaaacagaccccgggacaagggctcgaatggattggcgccatctaccccgggaatggcgatacttcgtacaaccagaagttcaagggaaaggccaccctgaccgccgacaagagctcctccaccgcgtatatgcagttgagctccctgacctccgaggactccgccgactactactgcgcacggtccaactactatggaagctcgtactggttcttcgatgtctggggggccggcaccactgtgaccgtcagctccgggggcggaggatccggtggaggcggaagcgggggtggaggatccgacattgtgctgactcagtccccggcaatcctgtcggcctcaccgggcgaaaaggtcacgatgacttgtagagcgtcgtccagcgtgaactacatggattggtaccaaaagaagcctggatcgtcacccaagccttggatctacgctacatctaacctggcctccggcgtgccagcgcggttcagcgggtccggctcgggcacctcatactcgctgaccatctcccgcgtggaggctgaggacgccgcgacctactactgccagcagtggtccttcaacccgccgacttttggaggcggtactaagctggagatcaaaggaggcggcggcagcggcgggggagggtccggagggggtggttctggtggaggaggatcgggaggcggtggcagcgacattcagatgactcagaccacctcctccctgtccgcctccctgggcgaccgcgtgaccatctcatgccgcgccagccaggacatctcgaagtacctcaactggtaccagcagaagcccgacggaaccgtgaagctcctgatctaccacacctcccggctgcacagcggagtgccgtctagattctcgggttcggggtcgggaactgactactcccttactatttccaacctggagcaggaggatattgccacctacttctgccaacaaggaaacaccctgccgtacacttttggcgggggaaccaagctggaaatcactggcagcacatccggttccgggaagcccggctccggagagggcagcaccaagggggaagtcaagctgcaggaatcaggacctggcctggtggccccgagccagtcactgtccgtgacttgtactgtgtccggagtgtcgctcccggattacggagtgtcctggatcaggcagccacctcggaaaggattggaatggctcggagtcatctggggttccgaaaccacctattacaactcggcactgaaatccaggctcaccattatcaaggataactccaagtcacaagtgttcctgaagatgaatagcctgcagactgacgacacggcgatctactattgcgccaagcactactactacggcggatcctacgctatggactactggggccaggggaccagcgtgaccgtgtcatccgcggccgcaactaccacccctgcccctcggccgccgactccggccccaaccatcgcaagccaacccctctccttgcgccccgaagcttgccgcccggccgcgggtggagccgtgcatacccgggggctggactttgcctgcgatatctacatttgggccccgctggccggcacttgcggcgtgctcctgctgtcgctggtcatcaccctttactgcaagaggggccggaagaagctgctttacatcttcaagcagccgttcatgcggcccgtgcagacgactcaggaagaggacggatgctcgtgcagattccctgaggaggaagaggggggatgcgaactgcgcgtcaagttctcacggtccgccgacgcccccgcatatcaacagggccagaatcagctctacaacgagctgaacctgggaaggagagaggagtacgacgtgctggacaagcgacgcggacgcgacccggagatgggggggaaaccacggcggaaaaaccctcaggaaggactgtacaacgaactccagaaagacaagatggcggaagcctactcagaaatcgggatgaagggagagcggaggaggggaaagggtcacgacgggctgtaccagggactgagcaccgccactaaggatacctacgatgccttgcatatgcaagcactcccaccccgg

SEQ ID NO: 26 - protein, 761 aa, synthetic construct
  REGION 1..761: note = LP-CD20 VH-(GGGGS)3-CD20 VL-(GGGGS)5-CD19VL-Whitlow linker-CD19 VH-CD8 hinge+TM-41BB-CD3zeta
MLLLVTSLLLCELPHPAFLLIPEVQLQQSGAELVKPGASVKMSCKASGYTFTSYNMHWVKQTPGQGLEWIGAIYPGNGDTSYNQKFKGKATLTADKSSSTAYMQLSSLTSEDSADYYCARSNYYGSSYWFFDVWGAGTTVTVSSGGGGSGGGGSGGGGSDIVLTQSPAILSASPGEKVTMTCRASSSVNYMDWYQKKPGSSPKPWIYATSNLASGVPARFSGSGSGTSYSLTISRVEAEDAATYYCQQWSFNPPTFGGGTKLEIKGGGGSGGGGSGGGGSGGGGSGGGGSDIQMTQTTSSLSASLGDRVTISCRASQDISKYLNWYQQKPDGTVKLLIYHTSRLHSGVPSRFSGSGSGTDYSLTISNLEQEDIATYFCQQGNTLPYTFGGGTKLEITGSTSGSGKPGSGEGSTKGEVKLQESGPGLVAPSQSLSVTCTVSGVSLPDYGVSWIRQPPRKGLEWLGVIWGSETTYYNSALKSRLTIIKDNSKSQVFLKMNSLQTDDTAIYYCAKHYYYGGSYAMDYWGQGTSVTVSSAAATTTPAPRPPTPAPTIASQPLSLRPEACRPAAGGAVHTRGLDFACDIYIWAPLAGTCGVLLLSLVITLYCKRGRKKLLYIFKQPFMRPVQTTQEEDGCSCRFPEEEEGGCELRVKFSRSADAPAYQQGQNQLYNELNLGRREEYDVLDKRRGRDPEMGGKPRRKNPQEGLYNELQKDKMAEAYSEIGMKGERRRGKGHDGLYQGLSTATKDTYDALHMQALPPR

SEQ ID NO: 27 - DNA, 726 bp, Mus musculus
  source 1..726: mol_type = other DNA
gacatccagatgacacagactacatcctccctgtctgcctctctgggagacagagtcaccatcagttgcagggcaagtcaggacattagtaaatatttaaattggtatcagcagaaaccagatggaactgttaaactcctgatctaccatacatcaagattacactcaggagtcccatcaaggttcagtggcagtgggtctggaacagattattctctcaccattagcaacctggagcaagaagatattgccacttacttttgccaacagggtaatacgcttccgtacacgttcggaggggggaccaagctggagatcacaggtggcggtggctcgggcggtggtgggtcgggtggcggcggatctgaggtgaaactgcaggagtcaggacctggcctggtggcgccctcacagagcctgtccgtcacatgcactgtctcaggggtctcattacccgactatggtgtaagctggattcgccagcctccacgaaagggtctggagtggctgggagtaatatggggtagtgaaaccacatactataattcagctctcaaatccagactgaccatcatcaaggacaactccaagagccaagttttcttaaaaatgaacagtctgcaaactgatgacacagccatttactactgtgccaaacattattactacggtggtagctatgctatggactactggggccaaggaacctcagtcaccgtctcctca

SEQ ID NO: 28 - protein, 242 aa, synthetic construct
  REGION 1..242: note = scFV for CD19
DIQMTQTTSSLSASLGDRVTISCRASQDISKYLNWYQQKPDGTVKLLIYHTSRLHSGVPSRFSGSGSGTDYSLTISNLEQEDIATYFCQQGNTLPYTFGGGTKLEITGGGGSGGGGSGGGGSEVKLQESGPGLVAPSQSLSVTCTVSGVSLPDYGVSWIRQPPRKGLEWLGVIWGSETTYYNSALKSRLTIIKDNSKSQVFLKMNSLQTDDTAIYYCAKHYYYGGSYAMDYWGQGTSVTVSS

SEQ ID NO: 29 - DNA, 1485 bp, synthetic construct
  misc_feature 1..1485: note = LP-CD19binder-CD8link-CD8tm-41BB-CD3zeta
  source 1..1485: mol_type = other DNA
atgcttctcctggtcacctccctgctcctctgcgaactgcctcaccctgccttccttctgattcctgacactgacattcagatgactcagaccacctcttccttgtccgcgtcactgggagacagagtgaccatctcgtgtcgcgcaagccaggatatctccaagtacctgaactggtaccaacagaagcccgacgggactgtgaagctgctgatctaccacacctcacgcctgcacagcggagtgccaagcagattctccggctccggctcgggaaccgattactcgcttaccattagcaacctcgagcaggaggacatcgctacctacttctgccagcaaggaaataccctgccctacaccttcggcggaggaaccaaattggaaatcaccggctccacgagcggctccgggaagcctggttccggggaaggctccactaagggtgaagtgaagctccaggagtccggccccggcctggtggcgccgtcgcaatcactctctgtgacctgtaccgtgtcgggagtgtccctgcctgattacggcgtgagctggattcggcagccgccgcggaagggcctggaatggctgggtgtcatctggggatccgagactacctactacaactcggccctgaagtcccgcctgactatcatcaaagacaactcgaagtcccaggtctttctgaagatgaactccctgcaaactgacgacaccgccatctattactgtgctaagcactactactacggtggaagctatgctatggactactggggccaggggacatccgtgacagtcagctccgcggccgcaactaccacccctgcccctcggccgccgactccggccccaaccatcgcaagccaacccctctccttgcgccccgaagcttgccgcccggccgcgggtggagccgtgcatacccgggggctggactttgcctgcgatatctacatttgggccccgctggccggcacttgcggcgtgctcctgctgtcgctggtcatcaccctttactgcaagaggggccggaagaagctgctttacatcttcaagcagccgttcatgcggcccgtgcagacgactcaggaagaggacggatgctcgtgcagattccctgaggaggaagaggggggatgcgaactgcgcgtcaagttctcacggtccgccgacgcccccgcatatcaacagggccagaatcagctctacaacgagctgaacctgggaaggagagaggagtacgacgtgctggacaagcgacgcggacgcgacccggagatgggggggaaaccacggcggaaaaaccctcaggaaggactgtacaacgaactccagaaagacaagatggcggaagcctactcagaaatcgggatgaagggagagcggaggaggggaaagggtcacgacgggctgtaccagggactgagcaccgccactaaggatacctacgatgccttgcatatgcaagcactcccaccccgg

SEQ ID NO: 30 - protein, 495 aa, synthetic construct
  REGION 1..495: note = LP-CD19binder-CD8link-CD8tm-41BB-CD3zeta
MLLLVTSLLLCELPHPAFLLIPDTDIQMTQTTSSLSASLGDRVTISCRASQDISKYLNWYQQKPDGTVKLLIYHTSRLHSGVPSRFSGSGSGTDYSLTISNLEQEDIATYFCQQGNTLPYTFGGGTKLEITGSTSGSGKPGSGEGSTKGEVKLQESGPGLVAPSQSLSVTCTVSGVSLPDYGVSWIRQPPRKGLEWLGVIWGSETTYYNSALKSRLTIIKDNSKSQVFLKMNSLQTDDTAIYYCAKHYYYGGSYAMDYWGQGTSVTVSSAAATTTPAPRPPTPAPTIASQPLSLRPEACRPAAGGAVHTRGLDFACDIYIWAPLAGTCGVLLLSLVITLYCKRGRKKLLYIFKQPFMRPVQTTQEEDGCSCRFPEEEEGGCELRVKFSRSADAPAYQQGQNQLYNELNLGRREEYDVLDKRRGRDPEMGGKPRRKNPQEGLYNELQKDKMAEAYSEIGMKGERRRGKGHDGLYQGLSTATKDTYDALHMQALPPR

SEQ ID NO: 31 - DNA, 1470 bp, synthetic construct
  misc_feature 1..1470: note = LP-CD19binder-CD8link-CD8tm-signals
  source 1..1470: mol_type = other DNA
atgcttctcctggtcacctccctgctcctctgcgaactgcctcaccctgccttccttctgattcctgacattcagatgactcagaccacctcttccttgtccgcgtcactgggagacagagtgaccatctcgtgtcgcgcaagccaggatatctccaagtacctgaactggtaccaacagaagcccgacgggactgtgaagctgctgatctaccacacctcacgcctgcacagcggagtgccaagcagattctccggctccggctcgggaaccgattactcgcttaccattagcaacctcgagcaggaggacatcgctacctacttctgccagcaaggaaataccctgccctacaccttcggcggaggaaccaaattggaaatcaccggcggaggaggctccgggggaggaggttccgggggcgggggttccgaagtgaagctccaggagtccggccccggcctggtggcgccgtcgcaatcactctctgtgacctgtaccgtgtcgggagtgtccctgcctgattacggcgtgagctggattcggcagccgccgcggaagggcctggaatggctgggtgtcatctggggatccgagactacctactacaactcggccctgaagtcccgcctgactatcatcaaagacaactcgaagtcccaggtctttctgaagatgaactccctgcaaactgacgacaccgccatctattactgtgctaagcactactactacggtggaagctatgctatggactactgggggcaaggcacttcggtgactgtgtcaagcgcggccgcaactaccacccctgcccctcggccgccgactccggccccaaccatcgcaagccaacccctctccttgcgccccgaagcttgccgcccggccgcgggtggagccgtgcatacccgggggctggactttgcctgcgatatctacatttgggccccgctggccggcacttgcggcgtgctcctgctgtcgctggtcatcaccctttactgcaagaggggccggaagaagctgctttacatcttcaagcagccgttcatgcggcccgtgcagacgactcaggaagaggacggatgctcgtgcagattccctgaggaggaagaggggggatgcgaactgcgcgtcaagttctcacggtccgccgacgcccccgcatatcaacagggccagaatcagctctacaacgagctgaacctgggaaggagagaggagtacgacgtgctggacaagcgacgcggacgcgacccggagatgggggggaaaccacggcggaaaaaccctcaggaaggactgtacaacgaactccagaaagacaagatggcggaagcctactcagaaatcgggatgaagggagagcggaggaggggaaagggtcacgacgggctgtaccagggactgagcaccgccactaaggatacctacgatgccttgcatatgcaagcactcccaccccgg

SEQ ID NO: 32 - protein, 490 aa, synthetic construct
  REGION 1..490: note = LP-CD19binder-CD8link-CD8tm-signals
MLLLVTSLLLCELPHPAFLLIPDIQMTQTTSSLSASLGDRVTISCRASQDISKYLNWYQQKPDGTVKLLIYHTSRLHSGVPSRFSGSGSGTDYSLTISNLEQEDIATYFCQQGNTLPYTFGGGTKLEITGGGGSGGGGSGGGGSEVKLQESGPGLVAPSQSLSVTCTVSGVSLPDYGVSWIRQPPRKGLEWLGVIWGSETTYYNSALKSRLTIIKDNSKSQVFLKMNSLQTDDTAIYYCAKHYYYGGSYAMDYWGQGTSVTVSSAAATTTPAPRPPTPAPTIASQPLSLRPEACRPAAGGAVHTRGLDFACDIYIWAPLAGTCGVLLLSLVITLYCKRGRKKLLYIFKQPFMRPVQTTQEEDGCSCRFPEEEEGGCELRVKFSRSADAPAYQQGQNQLYNELNLGRREEYDVLDKRRGRDPEMGGKPRRKNPQEGLYNELQKDKMAEAYSEIGMKGERRRGKGHDGLYQGLSTATKDTYDALHMQALPPR

SEQ ID NO: 33 - DNA, 1548 bp, synthetic construct
  misc_feature 1..1548: note = CD19_20-reactive scFv binding domain
  source 1..1548: mol_type = other DNA
gacattcagatgactcagaccacctcctccctgtccgcctccctgggcgaccgcgtgaccatctcatgccgcgccagccaggacatctcgaagtacctcaactggtaccagcagaagcccgacggaaccgtgaagctcctgatctaccacacctcccggctgcacagcggagtgccgtctagattctcgggttcggggtcgggaactgactactcccttactatttccaacctggagcaggaggatattgccacctacttctgccaacaaggaaacaccctgccgtacacttttggcgggggaaccaagctggaaatcactggcagcacatccggttccgggaagcccggctccggagagggcagcaccaagggggaagtcaagctgcaggaatcaggacctggcctggtggccccgagccagtcactgtccgtgacttgtactgtgtccggagtgtcgctcccggattacggagtgtcctggatcaggcagccacctcggaaaggattggaatggctcggagtcatctggggttccgaaaccacctattacaactcggcactgaaatccaggctcaccattatcaaggataactccaagtcacaagtgttcctgaagatgaatagcctgcagactgacgacacggcgatctactattgcgccaagcactactactacggcggatcctacgctatggactactggggccaggggaccagcgtgaccgtgtcatccggaggcggcggcagcggcgggggagggtccggagggggtggttctggtggaggaggatcgggaggcggtggcagcgaggtgcagttgcaacagtcaggagctgaactggtcaagccaggagccagcgtgaagatgagctgcaaggcctccggttacaccttcacctcctacaacatgcactgggtgaaacagaccccgggacaagggctcgaatggattggcgccatctaccccgggaatggcgatacttcgtacaaccagaagttcaagggaaaggccaccctgaccgccgacaagagctcctccaccgcgtatatgcagttgagctccctgacctccgaggactccgccgactactactgcgcacggtccaactactatggaagctcgtactggttcttcgatgtctggggggccggcaccactgtgaccgtcagctccgggggcggaggatccggtggaggcggaagcgggggtggaggatccgacattgtgctgactcagtccccggcaatcctgtcggcctcaccgggcgaaaaggtcacgatgacttgtagagcgtcgtccagcgtgaactacatggattggtaccaaaagaagcctggatcgtcacccaagccttggatctacgctacatctaacctggcctccggcgtgccagcgcggttcagcgggtccggctcgggcacctcatactcgctgaccatctcccgcgtggaggctgaggacgccgcgacctactactgccagcagtggtccttcaacccgccgacttttggaggcggtactaagctggagatcaaagcggccgca

SEQ ID NO: 34 - protein, 516 aa, synthetic construct
  REGION 1..516: note = CD19_20-reactive scFv binding domain
DIQMTQTTSSLSASLGDRVTISCRASQDISKYLNWYQQKPDGTVKLLIYHTSRLHSGVPSRFSGSGSGTDYSLTISNLEQEDIATYFCQQGNTLPYTFGGGTKLEITGSTSGSGKPGSGEGSTKGEVKLQESGPGLVAPSQSLSVTCTVSGVSLPDYGVSWIRQPPRKGLEWLGVIWGSETTYYNSALKSRLTIIKDNSKSQVFLKMNSLQTDDTAIYYCAKHYYYGGSYAMDYWGQGTSVTVSSGGGGSGGGGSGGGGSGGGGSGGGGSEVQLQQSGAELVKPGASVKMSCKASGYTFTSYNMHWVKQTPGQGLEWIGAIYPGNGDTSYNQKFKGKATLTADKSSSTAYMQLSSLTSEDSADYYCARSNYYGSSYWFFDVWGAGTTVTVSSGGGGSGGGGSGGGGSDIVLTQSPAILSASPGEKVTMTCRASSSVNYMDWYQKKPGSSPKPWIYATSNLASGVPARFSGSGSGTSYSLTISRVEAEDAATYYCQQWSFNPPTFGGGTKLEIKAAA

SEQ ID NO: 35 - DNA, 2283 bp, synthetic construct
  misc_feature 1..2283: note = LP-CD19 VL-Whitlow linker-CD19 VH (GGGGS)5 CD20 VH (GGGGS)3-CD20 VL CD8 hinge+TM-41BB-CD3zeta
  source 1..2283: mol_type = other DNA
atgctccttctcgtgacctccctgcttctctgcgaactgccccatcctgccttcctgctgattcccgacattcagatgactcagaccacctcctccctgtccgcctccctgggcgaccgcgtgaccatctcatgccgcgccagccaggacatctcgaagtacctcaactggtaccagcagaagcccgacggaaccgtgaagctcctgatctaccacacctcccggctgcacagcggagtgccgtctagattctcgggttcggggtcgggaactgactactcccttactatttccaacctggagcaggaggatattgccacctacttctgccaacaaggaaacaccctgccgtacacttttggcgggggaaccaagctggaaatcactggcagcacatccggttccgggaagcccggctccggagagggcagcaccaagggggaagtcaagctgcaggaatcaggacctggcctggtggccccgagccagtcactgtccgtgacttgtactgtgtccggagtgtcgctcccggattacggagtgtcctggatcaggcagccacctcggaaaggattggaatggctcggagtcatctggggttccgaaaccacctattacaactcggcactgaaatccaggctcaccattatcaaggataactccaagtcacaagtgttcctgaagatgaatagcctgcagactgacgacacggcgatctactattgcgccaagcactactactacggcggatcctacgctatggactactggggccaggggaccagcgtgaccgtgtcatccggaggcggcggcagcggcgggggagggtccggagggggtggttctggtggaggaggatcgggaggcggtggcagcgaggtgcagttgcaacagtcaggagctgaactggtcaagccaggagccagcgtgaagatgagctgcaaggcctccggttacaccttcacctcctacaacatgcactgggtgaaacagaccccgggacaagggctcgaatggattggcgccatctaccccgggaatggcgatacttcgtacaaccagaagttcaagggaaaggccaccctgaccgccgacaagagctcctccaccgcgtatatgcagttgagctccctgacctccgaggactccgccgactactactgcgcacggtccaactactatggaagctcgtactggttcttcgatgtctggggggccggcaccactgtgaccgtcagctccgggggcggaggatccggtggaggcggaagcgggggtggaggatccgacattgtgctgactcagtccccggcaatcctgtcggcctcaccgggcgaaaaggtcacgatgacttgtagagcgtcgtccagcgtgaactacatggattggtaccaaaagaagcctggatcgtcacccaagccttggatctacgctacatctaacctggcctccggcgtgccagcgcggttcagcgggtccggctcgggcacctcatactcgctgaccatctcccgcgtggaggctgaggacgccgcgacctactactgccagcagtggtccttcaacccgccgacttttggaggcggtactaagctggagatcaaagcggccgcaactaccacccctgcccctcggccgccgactccggccccaaccatcgcaagccaacccctctccttgcgccccgaagcttgccgcccggccgcgggtggagccgtgcatacccgggggctggactttgcctgcgatatctacatttgggccccgctggccggcacttgcggcgtgctcctgctgtcgctggtcatcaccctttactgcaagaggggccggaagaagctgctttacatcttcaagcagccgttcatgcggcccgtgcagacgactcaggaagaggacggatgctcgtgcagattccctgaggaggaagaggggggatgcgaactgcgcgtcaagttctcacggtccgccgacgcccccgcatatcaacagggccagaatcagctctacaacgagctgaacctgggaaggagagaggagtacgacgtgctggacaagcgacgcggacgcgacccggagatgggggggaaaccacggcggaaaaaccctcaggaaggactgtacaacgaactccagaaagacaagatggcggaagcctactcagaaatcgggatgaagggagagcggaggaggggaaagggtcacgacgggctgtaccagggactgagcaccgccactaaggatacctacgatgccttgcatatgcaagcactcccaccccgg

SEQ ID NO: 36 - protein, 761 aa, synthetic construct
  REGION 1..761: note = LP-CD19 VL-Whitlow linker-CD19 VH (GGGGS)5 CD20 VH (GGGGS)3-CD20 VL CD8 hinge+TM-41BB-CD3zeta
MLLLVTSLLLCELPHPAFLLIPDIQMTQTTSSLSASLGDRVTISCRASQDISKYLNWYQQKPDGTVKLLIYHTSRLHSGVPSRFSGSGSGTDYSLTISNLEQEDIATYFCQQGNTLPYTFGGGTKLEITGSTSGSGKPGSGEGSTKGEVKLQESGPGLVAPSQSLSVTCTVSGVSLPDYGVSWIRQPPRKGLEWLGVIWGSETTYYNSALKSRLTIIKDNSKSQVFLKMNSLQTDDTAIYYCAKHYYYGGSYAMDYWGQGTSVTVSSGGGGSGGGGSGGGGSGGGGSGGGGSEVQLQQSGAELVKPGASVKMSCKASGYTFTSYNMHWVKQTPGQGLEWIGAIYPGNGDTSYNQKFKGKATLTADKSSSTAYMQLSSLTSEDSADYYCARSNYYGSSYWFFDVWGAGTTVTVSSGGGGSGGGGSGGGGSDIVLTQSPAILSASPGEKVTMTCRASSSVNYMDWYQKKPGSSPKPWIYATSNLASGVPARFSGSGSGTSYSLTISRVEAEDAATYYCQQWSFNPPTFGGGTKLEIKAAATTTPAPRPPTPAPTIASQPLSLRPEACRPAAGGAVHTRGLDFACDIYIWAPLAGTCGVLLLSLVITLYCKRGRKKLLYIFKQPFMRPVQTTQEEDGCSCRFPEEEEGGCELRVKFSRSADAPAYQQGQNQLYNELNLGRREEYDVLDKRRGRDPEMGGKPRRKNPQEGLYNELQKDKMAEAYSEIGMKGERRRGKGHDGLYQGLSTATKDTYDALHMQALPPR

SEQ ID NO: 37 - DNA, 732 bp, synthetic construct
  misc_feature 1..732: note = mesothelin-reactive scFv binding domain
  source 1..732: mol_type = other DNA
gaggtccagctggtacagtctgggggaggcttggtacagcctggggggtccctgagactctcctgtgcagcctctggattcacctttgatgattatgccatgcactgggtccggcaagctccagggaagggcctggagtgggtctcaggtattagttggaatagtggtagcataggctatgcggactctgtgaagggccgattcaccatctccagagacaacgccaagaactccctgtatctgcaaatgaacagtctgagagctgaggacacggccttgtattactgtgcaaaagatttatcgtcagtggctggaccctttaactactggggccagggcaccctggtcaccgtctcctcaggaggtggcgggtctggtggaggcggtagcggcggtggcggatcctcttctgagctgactcaggaccctgctgtgtctgtggccttgggacagacagtcaggatcacatgccaaggagacagcctcagaagctattatgcaagctggtaccagcagaagccaggacaggcccctgtacttgtcatctatggtaaaaacaaccggccctcagggatcccagaccgattctctggctccagctcaggaaacacagcttccttgaccatcactggggctcaggcggaggatgaggctgactattactgtaactcccgggacagcagtggtaaccatctggtattcggcggaggcacccagctgaccgtcctcggt

SEQ ID NO: 38 - protein, 244 aa, synthetic construct
  REGION 1..244: note = mesothelin-reactive scFv binding domain
EVQLVQSGGGLVQPGGSLRLSCAASGFTFDDYAMHWVRQAPGKGLEWVSGISWNSGSIGYADSVKGRFTISRDNAKNSLYLQMNSLRAEDTALYYCAKDLSSVAGPFNYWGQGTLVTVSSGGGGSGGGGSGGGGSSSELTQDPAVSVALGQTVRITCQGDSLRSYYASWYQQKPGQAPVLVIYGKNNRPSGIPDRFSGSSSGNTASLTITGAQAEDEADYYCNSRDSSGNHLVFGGGTQLTVLG

SEQ ID NO: 39 - DNA, 1476 bp, synthetic construct
  misc_feature 1..1476: note = LP-LTG1904-CD8 TM-41BB-CD3zeta
  source 1..1476: mol_type = other DNA
atgctgctgctggtgaccagcctgctgctgtgcgaactgccgcatccggcgtttctgctgattccggaggtccagctggtacagtctgggggaggcttggtacagcctggggggtccctgagactctcctgtgcagcctctggattcacctttgatgattatgccatgcactgggtccggcaagctccagggaagggcctggagtgggtctcaggtattagttggaatagtggtagcataggctatgcggactctgtgaagggccgattcaccatctccagagacaacgccaagaactccctgtatctgcaaatgaacagtctgagagctgaggacacggccttgtattactgtgcaaaagatttatcgtcagtggctggaccctttaactactggggccagggcaccctggtcaccgtctcctcaggaggtggcgggtctggtggaggcggtagcggcggtggcggatcctcttctgagctgactcaggaccctgctgtgtctgtggccttgggacagacagtcaggatcacatgccaaggagacagcctcagaagctattatgcaagctggtaccagcagaagccaggacaggcccctgtacttgtcatctatggtaaaaacaaccggccctcagggatcccagaccgattctctggctccagctcaggaaacacagcttccttgaccatcactggggctcaggcggaggatgaggctgactattactgtaactcccgggacagcagtggtaaccatctggtattcggcggaggcacccagctgaccgtcctcggtgcggccgcaactaccacccctgcccctcggccgccgactccggccccaaccatcgcaagccaacccctctccttgcgccccgaagcttgccgcccggccgcgggtggagccgtgcatacccgggggctggactttgcctgcgatatctacatttgggccccgctggccggcacttgcggcgtgctcctgctgtcgctggtcatcaccctttactgcaagaggggccggaagaagctgctttacatcttcaagcagccgttcatgcggcccgtgcagacgactcaggaagaggacggatgctcgtgcagattccctgaggaggaagaggggggatgcgaactgcgcgtcaagttctcacggtccgccgacgcccccgcatatcaacagggccagaatcagctctacaacgagctgaacctgggaaggagagaggagtacgacgtgctggacaagcgacgcggacgcgacccggagatgggggggaaaccacggcggaaaaaccctcaggaaggactgtacaacgaactccagaaagacaagatggcggaagcctactcagaaatcgggatgaagggagagcggaggaggggaaagggtcacgacgggctgtaccagggactgagcaccgccactaaggatacctacgatgccttgcatatgcaagcactcccaccccgg

SEQ ID NO: 40 - protein, 492 aa, synthetic construct
  REGION 1..492: note = LP-LTG1904-CD8 TM-41BB-CD3zeta
MLLLVTSLLLCELPHPAFLLIPEVQLVQSGGGLVQPGGSLRLSCAASGFTFDDYAMHWVRQAPGKGLEWVSGISWNSGSIGYADSVKGRFTISRDNAKNSLYLQMNSLRAEDTALYYCAKDLSSVAGPFNYWGQGTLVTVSSGGGGSGGGGSGGGGSSSELTQDPAVSVALGQTVRITCQGDSLRSYYASWYQQKPGQAPVLVIYGKNNRPSGIPDRFSGSSSGNTASLTITGAQAEDEADYYCNSRDSSGNHLVFGGGTQLTVLGAAATTTPAPRPPTPAPTIASQPLSLRPEACRPAAGGAVHTRGLDFACDIYIWAPLAGTCGVLLLSLVITLYCKRGRKKLLYIFKQPFMRPVQTTQEEDGCSCRFPEEEEGGCELRVKFSRSADAPAYQQGQNQLYNELNLGRREEYDVLDKRRGRDPEMGGKPRRKNPQEGLYNELQKDKMAEAYSEIGMKGERRRGKGHDGLYQGLSTATKDTYDALHMQALPPR

SEQ ID NO: 41 - DNA, 339 bp, synthetic construct
  misc_feature 1..339: note = CD33-reactive single chain binding domain VH-4
  source 1..339: mol_type = other DNA
gaggtgcagctggtggagtctgggggaggcttggtacagcctggagggtccctgagactctcctgtgcagcctctggattcaccttcagtagctatggcatgagctgggtccgccaggctccaagacaagggcttgagtgggtggccaacataaagcaagatggaagtgagaaatactatgcggactcagtgaagggccgattcaccatctccagagacaattccaagaacacgctgtatctgcaaatgaacagcctgagagccgaggacacagccacgtattactgtgcgaaagaaaatgtggactggggccagggcaccctggtcaccgtctcctca

SEQ ID NO: 42 - protein, 113 aa, synthetic construct
  REGION 1..113: note = CD33-reactive single chain binding domain VH-4
EVQLVESGGGLVQPGGSLRLSCAASGFTFSSYGMSWVRQAPRQGLEWVANIKQDGSEKYYADSVKGRFTISRDNSKNTLYLQMNSLRAEDTATYYCAKENVDWGQGTLVTVSS

SEQ ID NO: 43 - DNA, 1083 bp, synthetic construct
  misc_feature 1..1083: note = LP-VH4-CD8 TM-41BB-CD3zeta
  source 1..1083: mol_type = other DNA
atgctgctgctggtgaccagcctgctgctgtgcgaactgccgcatccggcgtttctgctgattccggaggtgcagctggtggagtctgggggaggcttggtacagcctggagggtccctgagactctcctgtgcagcctctggattcaccttcagtagctatggcatgagctgggtccgccaggctccaagacaagggcttgagtgggtggccaacataaagcaagatggaagtgagaaatactatgcggactcagtgaagggccgattcaccatctccagagacaattccaagaacacgctgtatctgcaaatgaacagcctgagagccgaggacacagccacgtattactgtgcgaaagaaaatgtggactggggccagggcaccctggtcaccgtctcctcagcggccgcaactaccacccctgcccctcggccgccgactccggccccaaccatcgcaagccaacccctctccttgcgccccgaagcttgccgcccggccgcgggtggagccgtgcatacccgggggctggactttgcctgcgatatctacatttgggccccgctggccggcacttgcggcgtgctcctgctgtcgctggtcatcaccctttactgcaagaggggccggaagaagctgctttacatcttcaagcagccgttcatgcggcccgtgcagacgactcaggaagaggacggatgctcgtgcagattccctgaggaggaagaggggggatgcgaactgcgcgtcaagttctcacggtccgccgacgcccccgcatatcaacagggccagaatcagctctacaacgagctgaacctgggaaggagagaggagtacgacgtgctggacaagcgacgcggacgcgacccggagatgggggggaaaccacggcggaaaaaccctcaggaaggactgtacaacgaactccagaaagacaagatggcggaagcctactcagaaatcgggatgaagggagagcggaggaggggaaagggtcacgacgggctgtaccagggactgagcaccgccactaaggatacctacgatgccttgcatatgcaagcactcccaccccgg

SEQ ID NO: 44 - protein, 361 aa, synthetic construct
  REGION 1..361: note = LP-VH4-CD8 TM-41BB-CD3zeta
MLLLVTSLLLCELPHPAFLLIPEVQLVESGGGLVQPGGSLRLSCAASGFTFSSYGMSWVRQAPRQGLEWVANIKQDGSEKYYADSVKGRFTISRDNSKNTLYLQMNSLRAEDTATYYCAKENVDWGQGTLVTVSSAAATTTPAPRPPTPAPTIASQPLSLRPEACRPAAGGAVHTRGLDFACDIYIWAPLAGTCGVLLLSLVITLYCKRGRKKLLYIFKQPFMRPVQTTQEEDGCSCRFPEEEEGGCELRVKFSRSADAPAYQQGQNQLYNELNLGRREEYDVLDKRRGRDPEMGGKPRRKNPQEGLYNELQKDKMAEAYSEIGMKGERRRGKGHDGLYQGLSTATKDTYDALHMQALPPR

SEQ ID NO: 45 - DNA, 797 bp, synthetic construct
  misc_feature 1..797: note = TSLPR-reactive scFv binding domain
  source 1..797: mol_type = other DNA
atggcactgcccgtgaccgccctgcttctgccgcttgcacttctgctgcacgccgctaggccccaagtcaccctcaaagagtcagggccaggaatcctcaagccctcacagactctgtctcttacttgctcattcagcggattcagcctttccacctctggtatgggcgtggggtggattaggcaacctagcggaaaggggcttgaatggctggcccacatctggtgggacgacgacaagtactacaacccctcactgaagtcccagctcactatttccaaagatacttcccggaatcaggtgttcctcaagattacctctgtcgacaccgctgataccgccacttactattgttcacgcagaccgagaggtaccatggacgcaatggactactggggacagggcaccagcgtgaccgtgtcatctggcggtggagggtcaggaggtggaggtagcggaggcggtgggtccgacattgtcatgacccaggccgccagcagcctgagcgcttcactgggcgacagggtgaccatcagctgtcgcgcatcacaagatatctctaagtatcttaattggtaccagcaaaagccggatggaaccgtgaagctgctgatctactacacctcacggctgcattctggagtgcctagccgctttagcggatctgggtccggtactgactacagcctcaccattagaaaccttgaacaggaggacatcgcaacttatttctgccaacaggtctatactctgccgtggaccttcggcggaggtaccaaactggagattaagtccgg

SEQ ID NO: 46 - protein, 265 aa, synthetic construct
  REGION 1..265: note = TSLPR-reactive scFv binding domain
MALPVTALLLPLALLLHAARPQVTLKESGPGILKPSQTLSLTCSFSGFSLSTSGMGVGWIRQPSGKGLEWLAHIWWDDDKYYNPSLKSQLTISKDTSRNQVFLKITSVDTADTATYYCSRRPRGTMDAMDYWGQGTSVTVSSGGGGSGGGGSGGGGSDIVMTQAASSLSASLGDRVTISCRASQDISKYLNWYQQKPDGTVKLLIYYTSRLHSGVPSRFSGSGSGTDYSLTIRNLEQEDIATYFCQQVYTLPWTFGGGTKLEIKS

SEQ ID NO: 47 - DNA, 1170 bp, synthetic construct
  misc_feature 1..1170: note = LP-3G11-CD8 TM-41BB-CD3zeta
  source 1..1170: mol_type = other DNA
atggcactgcccgtgaccgccctgcttctgccgcttgcacttctgctgcacgccgctaggccccaagtcaccctcaaagagtcagggccaggaatcctcaagccctcacagactctgtctcttacttgctcattcagcggattcagcctttccacctctggtatgggcgtggggtggattaggcaacctagcggaaaggggcttgaatggctggcccacatctggtgggacgacgacaagtactacaacccctcactgaagtcccagctcactatttccaaagatacttcccggaatcaggtgttcctcaagattacctctgtcgacaccgctgataccgccacttactattgttcacgcagaccgagaggtaccatggacgcaatggactactggggacagggcaccagcgtgaccgtgtcatctggcggtggagggtcaggaggtggaggtagcggaggcggtgggtccgacattgtcatgacccaggccgccagcagcctgagcgcttcactgggcgacagggtgaccatcagctgtcgcgcatcacaagatatctctaagtatcttaattggtaccagcaaaagccggatggaaccgtgaagctgctgatctactacacctcacggctgcattctggagtgcctagccgctttagcggcacttgcggcgtgctcctgctgtcgctggtcatcaccctttactgcaagaggggccggaagaagctgctttacatcttcaagcagccgttcatgcggcccgtgcagacgactcaggaagaggacggatgctcgtgcagattccctgaggaggaagaggggggatgcgaactgcgcgtcaagttctcacggtccgccgacgcccccgcatatcaacagggccagaatcagctctacaacgagctgaacctgggaaggagagaggagtacgacgtgctggacaagcgacgcggacgcgacccggagatgggggggaaaccacggcggaaaaaccctcaggaaggactgtacaacgaactccagaaagacaagatggcggaagcctactcagaaatcgggatgaagggagagcggaggaggggaaagggtcacgacgggctgtaccagggactgagcaccgccactaaggatacctacgatgccttgcatatgcaagcactcccaccccgg

SEQ ID NO: 48 - protein, 490 aa, synthetic construct
  REGION 1..490: note = LP-3G11-CD8 TM-41BB-CD3zeta
MALPVTALLLPLALLLHAARPQVTLKESGPGILKPSQTLSLTCSFSGFSLSTSGMGVGWIRQPSGKGLEWLAHIWWDDDKYYNPSLKSQLTISKDTSRNQVFLKITSVDTADTATYYCSRRPRGTMDAMDYWGQGTSVTVSSGGGGSGGGGSGGGGSDIVMTQAASSLSASLGDRVTISCRASQDISKYLNWYQQKPDGTVKLLIYYTSRLHSGVPSRFSGSGSGTDYSLTIRNLEQEDIATYFCQQVYTLPWTFGGGTKLEIKAAATTTPAPRPPTPAPTIASQPLSLRPEACRPAAGGAVHTRGLDFACDIYIWAPLAGTCGVLLLSLVITLYCKRGRKKLLYIFKQPFMRPVQTTQEEDGCSCRFPEEEEGGCELRVKFSRSADAPAYQQGQNQLYNELNLGRREEYDVLDKRRGRDPEMGGKPRRKNPQEGLYNELQKDKMAEAYSEIGMKGERRRGKGHDGLYQGLSTATKDTYDALHMQALPPR

SEQ ID NO: 49 - DNA, 1467 bp, synthetic construct
  misc_feature 1..1467: note = LP-CD19-TNFRSF19TM-41BB-CD3zeta
  source 1..1467: mol_type = other DNA
atgctgctgctggtcaccagcctgctgctgtgcgagctccctcaccccgcctttctgcttatcccggacattcagatgacacagaccacctcgagcttgtccgcgtcgctgggcgatcgcgtgaccatctcctgccgggcctcccaagacatttcaaagtatctcaactggtaccagcagaagccggacggaaccgtgaaactgctgatctaccataccagccgcctgcactccggcgtgccgtcccgcttctccggatcgggttccggaactgactactcactgactatctccaacttggaacaagaggacatcgccacttacttctgtcaacaaggaaatacccttccctacaccttcggggggggtaccaagctggagatcactgggggcggaggctccggtggaggcggatccggcggtggagggagcgaagtcaagctgcaggaatcaggaccaggactcgtggcgccatcccagtccctgtcggtgacctgtactgtctccggagtcagcctccccgattacggagtgtcatggattaggcaacccccaagaaaagggctggaatggctcggagtgatctggggctccgaaaccacctactacaactcggcgctgaagtcccggctgaccatcatcaaggacaactccaagagccaagtgttcttgaagatgaacagcttgcagaccgacgataccgcaatctactactgtgccaagcactattactacggggggtcttacgccatggactactggggacagggcacctccgtgactgtgtcgtccgcggccgcgcccgcccctcggcccccgactcctgccccgacgatcgcttcccaacctctctcgctgcgcccggaagcatgccggcccgccgccggtggcgctgtccacactcgcggactggactttgataccgcactggcggccgtgatctgtagcgccctggccaccgtgctgctggcgctgctcatcctttgcgtgatctactgcaagcggcagcctaggcgaaagaagctcctctacattttcaagcaacccttcatgcgccccgtgcaaaccacccaggaggaggatggatgctcatgccggttccctgaggaagaagagggcggttgcgagctcagagtgaaattcagccggtcggctgacgccccggcgtaccagcagggccagaaccagctgtacaatgagctcaacctggggcgccgcgaagagtacgacgtgctggacaagaggagaggcagagatccggaaatgggcggaaagccaaggcggaagaacccgcaggaaggtctttacaacgaactgcagaaggacaagatggccgaggcctactccgagattgggatgaagggagaaagacggaggggaaagggacatgacggactttaccagggcctgagcactgccacgaaggacacctatgatgccctgcacatgcaggcgctgccgcctcgg

SEQ ID NO: 50 - protein, 489 aa, synthetic construct
  REGION 1..489: note = LP-CD19-TNFRSF19TM-41BB-CD3zeta
MLLLVTSLLLCELPHPAFLLIPDIQMTQTTSSLSASLGDRVTISCRASQDISKYLNWYQQKPDGTVKLLIYHTSRLHSGVPSRFSGSGSGTDYSLTISNLEQEDIATYFCQQGNTLPYTFGGGTKLEITGGGGSGGGGSGGGGSEVKLQESGPGLVAPSQSLSVTCTVSGVSLPDYGVSWIRQPPRKGLEWLGVIWGSETTYYNSALKSRLTIIKDNSKSQVFLKMNSLQTDDTAIYYCAKHYYYGGSYAMDYWGQGTSVTVSSAAAPAPRPPTPAPTIASQPLSLRPEACRPAAGGAVHTRGLDFDTALAAVICSALATVLLALLILCVIYCKRQPRRKKLLYIFKQPFMRPVQTTQEEDGCSCRFPEEEEGGCELRVKFSRSADAPAYQQGQNQLYNELNLGRREEYDVLDKRRGRDPEMGGKPRRKNPQEGLYNELQKDKMAEAYSEIGMKGERRRGKGHDGLYQGLSTATKDTYDALHMQALPPR

SEQ ID NO: 51 - DNA, 2280 bp, synthetic construct
  misc_feature 1..2280: note = LP-CD20_CD19-CD8TM-CD28-CD3zeta
  source 1..2280: mol_type = other DNA
atgctccttctcgtgacctccctgcttctctgcgaactgccccatcctgccttcctgctgattcccgaggtgcagttgcaacagtcaggagctgaactggtcaagccaggagccagcgtgaagatgagctgcaaggcctccggttacaccttcacctcctacaacatgcactgggtgaaacagaccccgggacaagggctcgaatggattggcgccatctaccccgggaatggcgatacttcgtacaaccagaagttcaagggaaaggccaccctgaccgccgacaagagctcctccaccgcgtatatgcagttgagctccctgacctccgaggactccgccgactactactgcgcacggtccaactactatggaagctcgtactggttcttcgatgtctggggggccggcaccactgtgaccgtcagctccgggggcggaggatccggtggaggcggaagcgggggtggaggatccgacattgtgctgactcagtccccggcaatcctgtcggcctcaccgggcgaaaaggtcacgatgacttgtagagcgtcgtccagcgtgaactacatggattggtaccaaaagaagcctggatcgtcacccaagccttggatctacgctacatctaacctggcctccggcgtgccagcgcggttcagcgggtccggctcgggcacctcatactcgctgaccatctcccgcgtggaggctgaggacgccgcgacctactactgccagcagtggtccttcaacccgccgacttttggaggcggtactaagctggagatcaaaggaggcggcggcagcggcgggggagggtccggagggggtggttctggtggaggaggatcgggaggcggtggcagcgacattcagatgactcagaccacctcctccctgtccgcctccctgggcgaccgcgtgaccatctcatgccgcgccagccaggacatctcgaagtacctcaactggtaccagcagaagcccgacggaaccgtgaagctcctgatctaccacacctcccggctgcacagcggagtgccgtctagattctcgggttcggggtcgggaactgactactcccttactatttccaacctggagcaggaggatattgccacctacttctgccaacaaggaaacaccctgccgtacacttttggcgggggaaccaagctggaaatcactggcagcacatccggttccgggaagcccggctccggagagggcagcaccaagggggaagtcaagctgcaggaatcaggacctggcctggtggccccgagccagtcactgtccgtgacttgtactgtgtccggagtgtcgctcccggattacggagtgtcctggatcaggcagccacctcggaaaggattggaatggctcggagtcatctggggttccgaaaccacctattacaactcggcactgaaatccaggctcaccattatcaaggataactccaagtcacaagtgttcctgaagatgaatagcctgcagactgacgacacggcgatctactattgcgccaagcactactactacggcggatcctacgctatggactactggggccaggggaccagcgtgaccgtgtcatccgcggccgcgactaccactcctgcaccacggccacctaccccagcccccaccattgcaagccagccactttcactgcgccccgaagcgtgtagaccagctgctggaggagccgtgcatacccgagggctggacttcgcctgtgacatctacatctgggccccattggctggaacttgcggcgtgctgctcttgtctctggtcattaccctgtactgccggtcgaagaggtccagactcttgcactccgactacatgaacatgactcctagaaggcccggacccactagaaagcactaccagccgtacgcccctcctcgggatttcgccgcataccggtccagagtgaagttcagccgctcagccgatgcaccggcctaccagcagggacagaaccagctctacaacgagctcaacctgggtcggcgggaagaatatgacgtgctggacaaacggcgcggcagagatccggagatggggggaaagccgaggaggaagaaccctcaagagggcctgtacaacgaactgcagaaggacaagatggcggaagcctactccgagatcggcatgaagggagaacgccggagagggaagggtcatgacggactgtaccagggcctgtcaactgccactaaggacacttacgatgcgctccatatgcaagctttgcccccgcgg

SEQ ID NO: 52 - protein, 760 aa, synthetic construct
  REGION 1..760: note = LP-CD20_CD19-CD8TM-CD28-CD3zeta
MLLLVTSLLLCELPHPAFLLIPEVQLQQSGAELVKPGASVKMSCKASGYTFTSYNMHWVKQTPGQGLEWIGAIYPGNGDTSYNQKFKGKATLTADKSSSTAYMQLSSLTSEDSADYYCARSNYYGSSYWFFDVWGAGTTVTVSSGGGGSGGGGSGGGGSDIVLTQSPAILSASPGEKVTMTCRASSSVNYMDWYQKKPGSSPKPWIYATSNLASGVPARFSGSGSGTSYSLTISRVEAEDAATYYCQQWSFNPPTFGGGTKLEIKGGGGSGGGGSGGGGSGGGGSGGGGSDIQMTQTTSSLSASLGDRVTISCRASQDISKYLNWYQQKPDGTVKLLIYHTSRLHSGVPSRFSGSGSGTDYSLTISNLEQEDIATYFCQQGNTLPYTFGGGTKLEITGSTSGSGKPGSGEGSTKGEVKLQESGPGLVAPSQSLSVTCTVSGVSLPDYGVSWIRQPPRKGLEWLGVIWGSETTYYNSALKSRLTIIKDNSKSQVFLKMNSLQTDDTAIYYCAKHYYYGGSYAMDYWGQGTSVTVSSAAATTTPAPRPPTPAPTIASQPLSLRPEACRPAAGGAVHTRGLDFACDIYIWAPLAGTCGVLLLSLVITLYCRSKRSRLLHSDYMNMTPRRPGPTRKHYQPYAPPRDFAAYRSRVKFSRSADAPAYQQGQNQLYNELNLGRREEYDVLDKRRGRDPEMGGKPRRKNPQEGLYNELQKDKMAEAYSEIGMKGERRRGKGHDGLYQGLSTATKDTYDALHMQALPPR

SEQ ID NO: 53 - protein, 18 aa, synthetic construct
GSTSGSGKPGSGEGSTKG

SEQ ID NO: 54 - protein, 15 aa, synthetic construct
GGGGSGGGGSGGGGS

SEQ ID NO: 55 - protein, 25 aa, synthetic construct
GGGGSGGGGSGGGGSGGGGSGGGGS